European Patent Application EP 4 166 154 A1, published April 19, 2023. Title: MAGNETIZED ELDERBERRY FERMENT FOR PREVENTING OSTEOPOROSIS AND IMPROVING IMMUNITY AND USE FOR ANTIOXIDATION BY THE SAME. Applicant: TCI CO., LTD. Application EP, filed September 28, 2022. The sequence listing filed with the application follows.

SEQUENCE LISTING (4 sequences)

SEQ ID NO: 1 - DNA, 23 bp, synthetic construct
  source 1..23: mol_type = other DNA
tcttcattgaccaaggaaatcgg

SEQ ID NO: 2 - DNA, 21 bp, synthetic construct
  source 1..21: mol_type = other DNA
tccggggtgcattatctctac

SEQ ID NO: 3 - DNA, 19 bp, synthetic construct
  source 1..19: mol_type = other DNA
ctgggctacactgagcacc

SEQ ID NO: 4 - DNA, 21 bp, synthetic construct
  source 1..21: mol_type = other DNA
aagtggtcgttgagggcaatg